European Patent Application EP 4 714 466 A1, published March 25, 2026. Title: 针对猫FIPV的多抗原mRNA疫苗开发. Applicant: 北京合生基因科技有限公司. The sequence listing filed with the application follows.

SEQUENCE LISTING (49 sequences)

SEQ ID NO: 1 - protein, 245 aa, synthetic construct
ERYCAMQNTGSQCINGTDSSCSTCFERGGLIWHLANWNFSWSVILIVFITVLKYGRPQFSWLVYGIKMLIMWLLWPIVLALTIFNAYSEYQVSRYVMFGFSVAGAVVTFALWMMYFVRSIQLYRRTKSWWSFNPETNAILCVNALGRSYVLPLDGTPTGVTLTLLSGNLYAEGFKMAGGLTIEHLPKYVMIATPSRTIVYTLVGKQLKATTATGWAYYVKSKAGDYSTEARTDNLSEHEKLLHMV

SEQ ID NO: 2 - protein, 375 aa, synthetic construct
ATQGQRVNWGDEPSKRRGRSNSRGRKNNTIPLSFFNPIQLEPGSKFWSVCPRDFVPKGIGNKDQQIGYWNRQERYRIVKGQRKELPERWFFYFLGTGPQADAKFKDKIDGVFWVAKDGAMNKPTTLGTRGTNNESKPLKFDGKIPPQFQLEVNRSRNNSRSGSQSRSVSRNRSQSRGRQQSNNQNNVEDTIVAVLQKLGVTEKQRSRSKSRDRGDSKPRDTTPNNANKHTWKKTAGKGDVTNFYGARSASANFGDSDLVANGNAAKSYPQIAECVPSVSSMLFGSQWSAEDDGDQVKVTLTHTYYLPKDDAKTSQFLEQIDAYKRPSQVAKDQRQRKSRSKSAEKKPEELSVTLVEAYTDVFDDTQVEMIDEVTN

SEQ ID NO: 3 - protein, 1433 aa, synthetic construct
TTNNECIQVNVTQLAGNENLIRDFLFSNFKEEGSVVVGGYYPTEVWYNCSRTARTTAFQYFNNIHAFYFVMEAMENSTGNARGKPLLFHVHGEPVSVIISAYRDDVQQRPLLKHGLVCITKNRHINYEQFTSNQWNSTCTGADRKIPFSVIPTDNGTKIYGLEWNDDFVTAYISGRSYHLNINTNWFNNVTLLYSRSSTATWEYSAAYAYQGVSNFTYYKLNNTNGLKTYELCEDYEHCTGYATNVFAPTSGGYIPDGFSFNNWFLLTNSSTFVSGRFVTNQPLLINCLWPVPSFGVAAQEFCFEGAQFSQCNGVSLNNTVDVIRFNLNFTADVQSGMGATVFSLNTTGGVILEISCYSDTVSESSSYSYGEIPFGITDGPRYCYVLYNGTALKYLGTLPPSVKEIAISKWGHFYINGYNFFSTFPIGCISFNLTTGVSGAFWTIAYTSYTEALVQVENTAIKNVTYCNSHINNIKCSQLTANLNNGFYPVASSEVGFVNKSVVLLPSFFTYTAVNITIDLGMKLSGYGQPIASTLSNITLPMQDNNTDVYCIRSNQFSVYVHSTCKSSLWDNIFNQDCTDVLEATAVIKTGTCPFSFDKLNNYLTFNKFCLSLSPVGANCKFDVAARTRTNEQVVRSLYVIYEEGDNIVGVPSDNSGLHDLSVLHLDSCTDYNIYGRTGVGIIRRTNSTLLSGLYYTSLSGDLLGFKNVSDGVIYSVTPCDVSAQAAVIDGAIVGAMTSINSELLGLTHWTTTPNFYYYSIYNYTSERTRDTAIDSNDVDCEPVITYSNIGVCKNGALVFINVTHSDGDVQPISTGNVTIPTNFTISVQVEYMQVYTTPVSIDCARYVCNGNPRCNKLLTQYVSACQTIEQALAMGARLENMEVDSMLFVSENALKLASVEAFNSTENLDSIYKEWPSIGGSWLGGLKDILPSHNSKRKYGSAIEDLLFDKVVTSGLGTVDEDYKRCTGGYDIADLVCAQYYNGIMVLPGVANADKMTMYTASLAGGITLGALGGGAVAIPFAVAVQARLNYVALQTDVLNKNQQILANAFNQAIGNITQAFGKVNDAIHQTSQGLATVAKALAKVQDVVNTQGQALSHLTVQLQNNFQAISSSISDIYNRLDPPSADAQVDRLITGRLTALNAFVSQTLTRQAEVRASRQLAKDKVNECVRSQSQRFGFCGNGTHLFSLANAAPNGMIFFHTVLLPTAYETVTAWSGICASDGDRTFGLVVKDVQLTLFRNLDDKFYLTPRTMYQPRVATSSDFVQIEGCDVLFVNATVIDLPSIIPDYIDINQTVQDILENYRPNWTVPEFTLDIFNATYLNLTGEIDDLEFRSEKLHNTTVELAILIDNINNTLVNLEWLNRIETYVKWPWYVWLLIGLVVVFCIPLLLFCCFSTGCCGCIGCLGSCCHSICSRRQFENYEPIEKVHVH

SEQ ID NO: 4 - DNA, 735 bp, synthetic construct
  source 1..735: mol_type = other DNA
gaacgctactgtgccatgcaaaatacaggctcgcagtgcattaatggcacagattcatcatgtagcacctgttttgaacgtggtggtcttatttggcatctggctaactggaacttcagctggtctgtaatattgattgtttttataacagtgttaaaatatggaagaccgcaattcagctggctcgtttatggcattaaaatgctgatcatgtggctattatggcctattgttctagcgcttacgatttttaatgcatactctgagtaccaagtttccagatatgtaatgttcggctttagtgttgcaggtgcagttgtaacgtttgcactatggatgatgtattttgtgagatctattcagctgtatagacggaccaaatcatggtggtcttttaatcctgaaaccaatgcgattctttgtgtcaatgcattgggtagaagctatgtactccctcttgatggcactcctacaggtgttactcttaccctactttcaggaaatctatacgctgaaggttttaaaatggctggtggtcttaccatcgagcatttgcctaaatatgtcatgattgctacgcctagtagaaccatcgtttacacattagttggaaaacaactaaaggcaactactgccactggatgggcttactatgtaaaatctaaagctggtgattactcaacagaagcacgtactgataatttgagtgaacatgaaaaattattacatatggtg

SEQ ID NO: 5 - DNA, 735 bp, synthetic construct
  source 1..735: mol_type = other DNA
gagagatactgtgccatgcagaacacaggcagccagtgcatcaatggaacagacagcagctgcagcacctgctttgaaagaggaggcctgatctggcacctggccaactggaacttcagctggagtgtgatcctgattgtcttcattacagtgctgaagtacggcaggccccagttcagctggctggtgtacggcatcaagatgctcatcatgtggctgctgtggcccattgtgttggccctcaccatcttcaatgcctacagcgagtaccaggtgtccagatacgtgatgttcggcttctcagtggcaggagccgtggtgacctttgccctctggatgatgtactttgtgaggtccatccagctctacagaagaacaaagagctggtggagcttcaacccagaaaccaacgccatcctgtgtgtcaatgccctgggcagatcctatgtgctgcccctggatggcacccccacaggcgtcaccctcaccctcctgagcggcaacctgtacgccgagggcttcaagatggccggcggcctgacaatcgagcacctgcccaagtatgtgatgattgccacccccagcaggacaatagtctacaccctggtgggaaaacagctgaaggctaccacagccacaggctgggcctactacgtcaagagcaaggccggcgactacagcacagaggccaggaccgacaacctgtccgaacatgaaaaactcctgcacatggtc

SEQ ID NO: 6 - DNA, 735 bp, synthetic construct
  source 1..735: mol_type = other DNA
gagaggtactgcgccatgcagaacacaggctcccagtgcatcaacggaacagactcctcctgcagcacctgcttcgagagaggaggcctcatttggcacctggccaactggaacttcagctggtcagtcattctgatagtcttcataacagtgctgaagtacggcaggccccagttctcctggctcgtgtatggcatcaagatgctgatcatgtggctgctgtggcccatcgtcctggccctgaccatcttcaacgcctactcagagtaccaggtcagcaggtacgtgatgttcggcttctccgtggccggagcagtggtgaccttcgccctgtggatgatgtacttcgtgaggagcatccaactgtacaggaggaccaaaagctggtggtccttcaacccagaaaccaacgccatcctctgcgtgaacgccctgggcaggtcctacgtcctccccctggacggcacccccaccggggtcaccctcaccctcctgtcagggaacctgtacgctgagggcttcaagatggctggaggcctgacaattgaacacctgcccaagtacgtcatgatcgcaacaccctccagaaccatcgtctacaccctggtgggcaagcagctgaaggccaccaccgccaccggctgggcctactacgtcaagtccaaggccggcgactacagcaccgaggccaggaccgacaacctctcagagcacgagaagctgctgcacatggtg

SEQ ID NO: 7 - DNA, 735 bp, synthetic construct
  source 1..735: mol_type = other DNA
gagaggtactgtgccatgcagaacaccggttcccagtgcatcaacggcacagactcctcctgctccacctgcttcgagagaggaggcctgatctggcacctggcaaactggaacttcagctggagcgtgatcctgatagtgttcataaccgtcctgaagtacggcagaccacagttctcatggcttgtctatggcatcaagatgctgattatgtggctgctttggcctatcgtcctggccctgaccatcttcaacgcctactctgagtaccaggtgtcaaggtatgtcatgttcggcttctcagtggctggagctgtggtgacctttgctctgtggatgatgtacttcgtgaggtccatccagctgtacaggaggacaaagtcatggtggtccttcaacccagaaaccaatgccatcctgtgcgtcaacgcactgggcagaagctacgtcctaccactggacggcactcctacaggagtgaccctgaccctgctgtcaggcaatctgtacgcagaggggttcaagatggccggtggcctgaccatcgagcatctgcctaagtacgtgatgatcgccacccctagcaggacaatcgtgtacaccctggtgggaaagcagctaaaggcgaccacagccacaggctgggcctactacgtgaagtccaaggcaggggactattcaaccgaggccaggaccgacaacctgtcagagcacgagaagctgctgcacatggtc

SEQ ID NO: 8 - DNA, 1125 bp, synthetic construct
  source 1..1125: mol_type = other DNA
gccacacagggacaacgcgtcaactggggagatgaaccttccaaaagacgtggtcgttctaactctcgtggtcggaagaataacactatacctctttcattcttcaatcccatccaactcgaaccaggatcaaaattttggagcgtatgtccgagagattttgttcccaagggaataggtaacaaggatcaacaaattggttattggaatagacaagagcgttaccgcattgtcaaaggtcagcgtaaggaacttcctgagaggtggtttttctacttcttaggcacaggacctcaagctgatgctaaatttaaagacaagattgatggagtcttctgggttgcaaaggatggtgccatgaataaaccaacaacacttggcactcgtggtaccaacaatgaatccaaaccactgaaatttgatggtaagataccaccgcaatttcagcttgaagtgaaccgatctaggaacaactcaagaagtggttctcagtctagatctgtctctagaaacaggtctcaatccagaggaagacaacaatccaataatcagaataatgttgaggatacaattgtagctgtgcttcagaaattaggtgttactgaaaagcaaaggtcacgttctaaatctagagatcgtggtgactctaaacctagagacacaacacctaataatgccaacaaacacacctggaagaagactgcaggtaaaggtgatgtgacaaatttctatggtgctagaagtgcttcagctaactttggtgatagtgatctcgttgccaacggtaacgctgccaaatcctaccctcagatagctgaatgcgttccatcagtgtctagcatgctcttcggtagtcaatggtctgctgaagatgatggtgatcaagtgaaagtcacgctcactcatacctattacctgccaaaagatgatgccaaaaccagccaattcctagaacagattgacgcttacaagcggccatctcaagtggctaaagatcagaggcaaagaaaatctcgttctaagtctgctgagaagaagcctgaggaattgtctgtaactcttgtagaggcatatacggatgtgtttgatgacacacaggttgagatgattgatgaggttacgaac

SEQ ID NO: 9 - DNA, 1125 bp, synthetic construct
  source 1..1125: mol_type = other DNA
gccacacagggccagagggtgaactggggcgacgagccatccaagaggaggggaaggagcaacagcagaggaaggaagaacaacaccatccccctgtccttcttcaacccaattcagctagagccaggcagcaagttctggtcagtgtgccccagagacttcgtgcccaagggcatcggaaacaaggaccagcagatcggctactggaacagacaggagagatacagaattgtgaaaggccagagaaaggagctgccagagaggtggttcttctacttcctgggcaccggcccacaggcagacgccaagttcaaggacaagatcgatggagtgttctgggtggccaaggacggcgccatgaacaagcccaccacactgggcacaagaggaacaaacaatgagagcaagccactgaagtttgatggcaagatcccaccccagttccagctggaggtgaacaggagcagaaacaacagcagaagcggcagccagagcagaagtgtgagcagaaacagaagccagagcagaggaagacagcagagcaacaaccagaacaacgtggaggacaccatcgtggccgtgctgcagaagctgggggtcacagaaaagcagaggagcagaagcaagagcagggacagaggagacagcaagccaagagacaccacccccaacaacgccaacaagcacacctggaagaagacagccggcaagggagatgtgaccaacttctacggcgccagaagcgccagcgccaacttcggagactcagacctggtggccaatggaaacgcagccaagagctacccccagatcgcagagtgtgtgccctctgtctccagcatgctgtttggcagccagtggagcgccgaggacgacggtgaccaggtgaaggtgaccctgacacacacatactacctgcccaaagatgacgccaagaccagccagttcctggagcagattgatgcctacaagaggcccagccaggtggccaaggaccagagacagaggaagagcaggtccaagagcgccgagaagaagccagaagaattgagtgtcaccctggtggaggcctacacagacgtgtttgatgacacccaggtggagatgattgatgaggtgaccaac

SEQ ID NO: 10 - DNA, 1125 bp, synthetic construct
  source 1..1125: mol_type = other DNA
gccacccagggccagagagtgaactggggcgacgagccctcaaaaaggaggggcagatccaacagcagaggcaggaagaacaacaccatccccctgagcttcttcaaccccatccagctggagccaggctccaagttctggtcagtgtgcccaagggacttcgtgcccaagggcatcggcaacaaggaccagcagatcggctactggaacaggcaggagagatacagaatcgtgaagggccagaggaaggaactgccagaaaggtggttcttctacttcctgggcaccggcccccaggctgacgccaagttcaaagacaagatcgacggggtgttctgggtggccaaggacggcgccatgaacaagccaacaacactgggcaccagaggaaccaacaacgagagcaagccactgaagtttgacggcaagatccccccccagttccagctggaagtcaacaggagcaggaacaacagcaggtccggctcacaaagcaggagcgtgtccagaaacagatcccagtcaagaggaagacagcagtccaacaaccagaacaacgtggaggacaccatagtggccgtgctgcagaagctgggagtcacagagaagcagaggagcagatccaagtccagggacaggggagacagcaagcccagggacaccacacccaacaacgccaacaagcacacctggaagaagacagccggcaagggagatgtgaccaacttctacggcgccagaagcgcctcagccaacttcggagactcagacctggtggccaacggaaacgccgccaagagctacccccagatcgccgaatgtgtcccctcagtgtcctccatgctcttcggctcacagtggtcagcagaggacgacggcgaccaggtgaaggtgaccctgacccacacctactacctgcccaaggacgacgccaagacaagccagttcctggagcagatcgacgcctacaagaggccatcccaggtggccaaggaccagaggcagaggaagagcagaagcaagtcagccgagaagaaaccagaggagctgtcagtcaccctggtggaggcctacaccgacgtgttcgacgacacccaggtggagatgatcgacgaggtgaccaac

SEQ ID NO: 11 - DNA, 1125 bp, synthetic construct
  source 1..1125: mol_type = other DNA
gcaacacaaggacagagagtaaattggggggatgagcccagcaagaggcgaggcagaagcaactcaagagggagaaaaaacaataccatcccactgtcattcttcaaccccattcaactggagccaggctctaaattctggagtgtatgccccagggactttgtgcccaagggcatagggaacaaggaccagcaaataggatactggaaccggcaggagagatacagaattgtcaagggtcagagaaaggagctgccagagagatggttcttctacttcctaggaacaggcccacaggcagacgctaagttcaaggataagatcgatggtgtcttctgggtcgccaaggatggtgcaatgaataaaccaaccaccctggggaccagggggacaaacaatgagtccaagcccctcaagtttgatggcaaaatccccccacagttccagctggaggtcaacaggagcaggaacaatagccgttcagggtcccagtccagatctgtgtccagaaacaggtcccagagcaggggacggcagcagagtaacaaccagaataatgtggaagacaccatagtagcagtgctccagaaactgggggtcacagaaaaacagaggagcaggtccaagtctagggaccgtggggactctaagccaagggacaccacacccaacaacgccaacaagcacacatggaaaaaaacagcagggaagggtgatgtcaccaacttttacggggccaggtcagcctctgcaaacttcggggatagtgacctggtggccaacggcaatgctgctaaatcctaccctcagattgctgagtgcgtaccctctgtatcctctatgctctttggctcacaatggtctgctgaggatgatggtgaccaggtcaaggtcaccttgacccatacctactatctgcccaaggatgatgcaaaaaccagccagttcctagagcagatagatgcctacaagaggcccagccaggtggccaaggatcagaggcagagaaagagcagatccaagagcgcagaaaagaaaccagaggagttatctgtgaccctggtggaggcctacacagatgtctttgatgatacacaggtggaaatgatagatgaggtgactaac

SEQ ID NO: 12 - DNA, 4302 bp, synthetic construct
  source 1..4302: mol_type = other DNA
acaacaaataatgaatgcatacaagttaacgtaacacaattggctggcaatgaaaaccttatcagagattttctgtttagtaactttaaagaagaaggaagtgtagttgttggtggttattaccctacagaggtgtggtacaactgctctagaacagctcgaactactgcctttcagtattttaataatatacatgccttttattttgttatggaagccatggaaaatagcactggtaatgcacgtggtaaaccattattatttcatgtgcatggtgagcctgttagtgttattatatcggcttatagggatgatgtgcaacaaaggccccttttaaaacatgggttagtgtgcataactaaaaatcgccatattaactatgaacaattcacctccaaccagtggaattccacatgtacgggtgctgacagaaaaattcctttctctgtcatacccacggacaatggaacaaaaatctatggtcttgagtggaatgatgactttgttacagcttatattagtggtcgttcttatcacttgaacatcaatactaattggtttaacaatgtcacacttttgtattcacgctcaagcactgctacctgggaatacagtgctgcatatgcttaccaaggtgtttctaacttcacttattacaagttaaataacaccaatggtctaaaaacctatgaattatgtgaagattatgaacattgcactggctatgctaccaatgtatttgctccgacatcaggtggttacatacctgatggatttagttttaacaattggttcttgcttacaaatagttccacttttgttagtggcaggtttgtaacaaatcaaccattattgattaattgcttgtggccagtgcccagttttggtgtagcagcacaagaattttgttttgaaggtgcacagtttagccaatgtaatggtgtgtctttaaataacacagtggatgttattagattcaaccttaatttcactgcagatgtacaatctggtatgggtgctacagtattttcactgaatacaacaggtggtgtcattcttgaaatttcatgttatagtgacacagtgagtgagtctagttcttacagttatggtgaaatcccgttcggcataactgacggaccacgatactgttatgtactttacaatggcacagctcttaaatatttaggaacattaccacccagtgtaaaggaaattgctattagtaagtggggccatttttatattaatggttacaatttctttagcacatttcctattggttgtatatcttttaatttaaccactggtgttagtggagctttttggacaattgcttacacatcgtatactgaagcattagtacaagttgaaaacacagctattaaaaatgtgacgtattgtaacagtcacattaataacattaaatgttctcaacttactgctaatttgaataatggattttatcctgttgcttcaagtgaagtaggtttcgttaataagagtgttgtgttattacctagctttttcacatacaccgctgtcaatataaccattgatcttggtatgaagcttagtggttatggtcaacccatagcctcgacactaagtaacatcacactaccaatgcaggataacaatactgatgtgtactgtattcgttctaaccaattctcagtttatgttcattccacttgcaaaagttctttatgggacaatatttttaatcaagactgcacggatgttttagaggctacagctgttataaaaactggtacttgtcctttctcatttgataaattgaacaattacttgacttttaacaagttctgtttgtcgttgagtcctgttggtgctaattgcaagtttgatgttgctgcacgtacaagaaccaatgagcaggttgttagaagtctatatgtaatatatgaagaaggagacaacatagtgggtgtaccgtctgataatagcggtctgcacgatttgtctgtgctacacctagactcctgtacagattacaatatatatggtagaactggtgttggtattattagacgaactaacagtacgctacttagtggcttatattacacatcactatcaggtgatttgttaggctttaaaaatgttagtgatggtgtcatttattctgtgacgccatgtgatgtaagcgcacaagcggctgttattgatggtgccatagttggagctatgacttccattaacagtgaactgttaggtctaacacattggacaacgacacctaatttttattactactctatatataattacacaagtgagaggactcgtggcactgcaattgacagtaacgatgttgattgtgaacctgtcataacctattctaatataggtgtttgtaaaaatggtgctttggtttttattaacgtcacacattctgacggagacgtgcaaccaattagcactggtaatgtcacgatacctacaaattttactatatctgtgcaagttgaatacatgcaggtttacactacaccagtatcaatagattgtgcaagatacgtttgtaatggtaaccctagatgtaacaaattgttaacacaatatgtgtctgcatgtcaaactattgaacaagcacttgcaatgggtgccagacttgaaaacatggaggttgattccatgttgtttgtctcggaaaatgcccttaaattggcatctgttgaggcgttcaatagtacagaaaatttagatcctatttacaaagaatggcctagcataggtggttcttggctaggaggtctaaaagatatactaccgtcccataatagcaaacgtaagtatggttctgctatagaagatttgctttttgataaagttgtaacatctggtttaggtacagttgatgaagattataaacgttgtactggtggttacgacatagcagacttggtgtgtgctcaatattacaatggcatcatggttctaccaggtgtagctaatgctgacaagatgactatgtacacagcatcacttgcaggtggtataacattaggtgcacttggtggtggcgccgtggctataccttttgcagtagcagtacaggctagacttaattatgttgctctacaaactgatgtattgaataaaaaccaacagatcctggctaatgctttcaatcaagctattggtaacattacacaggcttttggtaaggttaatgatgctatacatcaaacatcacaaggtcttgccactgttgctaaagcgttggcaaaagtgcaagatgttgtcaacacacaagggcaagctttaagtcaccttacagtacaattgcaaaataattttcaagccattagtagttctattagtgatatttataacaggcttgacgaactgagtgctgatgcacaagttgataggctgattacaggtagacttacagcacttaatgcatttgtgtctcagactctaaccagacaagcagaggttagggctagtagacaacttgccaaagacaaggttaatgaatgtgttaggtctcagtctcagagattcggattctgtggtaatggtacacatttgttttcactagcaaatgcagcaccaaatggcatgattttctttcatacagtactattaccaacagcttatgaaactgtaacagcttggtcaggtatttgtgcttcagatggcgatcgcactttcggacttgtcgttaaagatgtgcagttgacgttgtttcgtaatctagatgacaagttctatttgacccccagaactatgtatcagcctagagttgcaactagttctgattttgttcaaattgaagggtgtgatgtgttgtttgtcaacgcgactgtaattgatttgcctagtattatacctgactatattgacattaatcaaactgttcaagacatattagaaaattacagaccaaactggactgtacctgaatttacacttgatattttcaacgcaacctatttaaatctgactggtgaaattgatgacttagagtttaggtcagaaaagctacataacactacagtagaacttgccattctcattgataacattaataatacattagtcaatcttgaatggctcaatagaattgaaacttatgtaaaatggccttggtatgtgtggctactgataggtttagtagtagtattttgcataccattactgctattttgctgttttagcacaggttgttgtggatgcataggttgtttaggaagttgttgtcactctatatgtagtagaagacaatttgaaaattatgaaccaattgaaaaagtgcatgtccactaa

SEQ ID NO: 13 - DNA, 4299 bp, synthetic construct
  source 1..4299: mol_type = other DNA
accaccaacaatgaatgcatccaggtgaacgtgacccagctggcaggcaatgaaaatttgatcagagacttcctgttcagcaacttcaaggaggagggcagtgtagtggtgggaggctactacccaacagaggtgtggtacaactgcagcagaacagccagaaccacagccttccagtacttcaacaacatccacgccttctactttgtgatggaggccatggaaaacagcacaggaaatgccagaggaaaacccctgctcttccacgtgcacggagagcccgtgtcagtcatcatcagcgcctacagagatgacgtccagcagcggcccctgctgaagcatggactggtctgcatcaccaagaacagacacatcaactacgagcagttcaccagcaaccagtggaacagcacctgcacaggagcagacagaaaaatccccttcagcgtcatccccacagacaacggcaccaaaatctatggcctggagtggaatgatgactttgtgacagcctatatcagcggcaggagctaccacctcaacatcaacaccaactggttcaacaacgtcaccctgctctactccagatccagcacagccacctgggagtacagcgccgcctatgcctaccagggagtctccaacttcacctactacaaactgaacaacaccaacggcctgaaaacctacgagctgtgtgaggactacgagcactgcacaggctatgccacaaatgtgtttgccccaaccagcggaggctacatcccagacggcttctccttcaacaactggttcctcctcaccaactcctccacatttgtgagcggcagatttgtgaccaaccagcccctgctgatcaactgcctgtggcccgtgcccagctttggagtggcagcccaggagttctgcttcgagggagcccagttcagccagtgcaacggagtcagcctgaacaacacagtggacgtgatcagattcaacctgaacttcacagcagacgtgcagagtggaatgggagccaccgtcttcagcctgaacaccacaggaggagtgatcctggagatcagctgctacagcgacacagtgagcgagagcagcagctacagctacggagagatcccatttggcatcacagatggccccaggtactgctacgtcctgtacaatggaacagccctgaaatacctgggcaccctcccacccagcgtgaaggagatcgccatcagcaagtggggccacttctacatcaatggctacaacttcttcagcaccttccccatcggctgcatctccttcaacctgaccacaggagtgagcggggccttctggacaatcgcctacacatcctacacagaagccctggtgcaggtggagaacacagccatcaaaaacgtcacctactgcaacagccacatcaacaacatcaagtgcagccagctgacagccaacctgaacaacggcttctacccagtggccagctcagaggtgggcttcgtgaacaagagcgtggtgctcctgcccagcttcttcacctacacagcagtgaacatcacaattgacctgggcatgaagctgagcggctacggccagccaattgccagcaccctctccaacatcaccctccccatgcaggacaataacacagatgtgtactgcatcagatccaaccagttctctgtctacgtgcacagcacctgcaaaagcagcctgtgggacaacatcttcaaccaggactgcacagatgtcctggaggccacagccgtgatcaaaacaggcacctgccccttcagctttgacaaactcaacaactaccttacattcaacaaattctgcctctccctcagcccagtgggagccaactgcaagtttgatgtggccgccaggaccaggacaaatgaacaagtggtcagaagcctctacgtcatctacgaggagggagacaacatcgtgggggtccccagcgacaacagcggcctgcacgacctgagtgtgctccacctggacagctgcacagactacaacatctacggcaggactggggtgggcatcatcagaagaaccaacagcacactgctgagtggcctgtactacaccagcctgagtggagacttgctgggcttcaagaatgtgtcagatggggtgatctacagtgtgaccccctgtgacgtgtctgcccaggctgcagtcatcgacggagccatcgtgggagccatgaccagcattaacagcgagctgctgggcctgacccactggaccaccacccccaacttctactactactccatctacaactacacatcagaaagaacaagagacacagccatcgacagcaatgacgtggactgtgagccagtcatcacctacagcaacatcggagtgtgcaagaacggagccctggtgttcatcaacgtgacccacagcgacggagatgtccagcccatcagcacaggaaatgtgaccatcccaaccaacttcaccatcagcgtccaggtggaatacatgcaggtgtacaccaccccagtgtccatcgactgtgccagatacgtgtgcaatggaaaccccagatgcaacaagctcctcacccagtacgtgtcagcctgccagacaatcgagcaggccctggccatgggagccaggctcgagaacatggaagtggacagcatgctgtttgtctcagagaatgccctgaaactggccagcgtggaggccttcaacagcacagagaacctggacagcatctacaaggagtggccatcaatcggaggcagctggctgggaggacttaaggacatcctgccaagccacaacagcaaaagaaagtacggcagcgccattgaggacctgctgtttgacaaggtggtcacctccggcctgggcacagtggatgaggactacaagagatgcaccggcggctatgacattgccgacctggtgtgtgcccagtactacaatggcatcatggtgctgcctggagtggccaacgccgacaaaatgaccatgtacaccgcctccctggctggaggcatcacactgggagccctggggggaggagcagtggccatcccctttgcagtggctgtgcaggccagactcaactacgtggccctgcagacagacgtgctcaacaagaaccagcagatcctggccaacgctttcaaccaggctatcggaaacatcacccaggcctttggaaaagtgaatgatgccatccaccagaccagccagggcctggccacagtggccaaggccctggccaaggtgcaggacgtggtcaacacccagggccaggccctcagtcacctcacagtacagctccagaacaacttccaggcaatctcctcctccatcagcgacatctacaacaggctggaccccccaagcgctgatgcccaggtggacagactgatcacaggaagactcacagccctcaacgcatttgtgtcccagacactgaccaggcaggcagaggtcagggccagcaggcagctggccaaggacaaggtgaatgagtgcgtgaggagccagagccagagatttggcttctgcggaaacggcacccacctgttcagcctggccaacgccgcccccaacggcatgattttcttccacacagtcctcctccccacagcctacgaaacagtgacagcctggtcaggcatctgtgccagcgacggagacagaacctttggcctggtggtgaaggatgtgcagctcaccctcttcagaaacctggatgacaagttctacctcaccccaagaaccatgtaccagcccagagtggccacaagcagcgactttgtgcagattgagggctgtgacgtgctgtttgtgaatgcaacagtgattgacctcccaagcatcatcccagattacatcgacatcaaccagacagtgcaggacatcctggagaactacaggcccaactggacagtgccagagttcaccctggacatcttcaacgccacctacctgaacctgacaggagaaattgacgacctggagttcagatcagaaaaacttcacaacaccaccgtggagcttgccatcctcattgacaacattaacaacacactggtcaacctggaatggctgaacagaattgaaacctacgtgaagtggccctggtatgtgtggctgctgattggactggtggtggtgttctgcatcccactgctgctgttctgctgcttcagcaccggctgctgtggatgcatcggctgcttgggcagctgctgccacagcatctgcagcaggaggcagtttgagaactacgaaccaattgaaaaagtgcacgtccac

SEQ ID NO: 14 - DNA, 4299 bp, synthetic construct
  source 1..4299: mol_type = other DNA
accaccaacaacgagtgcatccaggtgaacgtgacccagctggcaggcaacgagaacctcatcagagacttcctcttctccaacttcaaggaggagggctcagtggtggtcggcggctactacccaacagaggtgtggtacaactgctcaaggaccgccagaaccacagccttccagtacttcaacaacatccacgccttctacttcgtgatggaggccatggagaactccaccgggaacgccaggggcaagccactactcttccacgtgcacggagagccagtgagcgtgatcatctcagcctacagggacgacgtgcagcagcgccccctgctgaagcatggactggtgtgcatcaccaagaacaggcacatcaactacgagcagttcaccagcaaccagtggaacagcacctgcaccggcgcagacaggaagatccccttctcagtgatcccaacagacaacggaaccaaaatctacggcctggagtggaacgacgacttcgtgaccgcctacatcagcggcaggtcctaccatctcaacatcaacaccaactggttcaacaacgtcaccctcctctacagcaggtcatccacagccacctgggagtactcagctgcctatgcataccagggagtctccaacttcacatactacaaactcaacaacaccaacggcctcaagacctacgagctgtgtgaggactacgagcactgcaccggctacgcaacaaacgtcttcgccccaacctccggaggctacatcccagacggcttctccttcaacaactggttcctcctcacaaacagctccaccttcgtgtcaggaaggttcgtgaccaaccagcccctgctcatcaactgcctctggcccgtcccctccttcggagtggccgcccaggagttctgcttcgagggagcccagttctcccagtgcaacggagtctccctcaacaacaccgtggacgtcatcagattcaacctcaacttcacagcagacgtccagagcggcatgggagccaccgtgttcagcctgaacaccacaggaggagtgatcctggagatctcctgctactcagacacagtgtcagagtcctcctcctacagctacggagagatcccattcggcatcacagacggccccagatactgctacgtgctgtacaacggcacagccctgaagtacctgggcaccctccccccatcagtgaaggagatcgccatcagcaagtggggccacttctacatcaacggctacaacttcttctccaccttccccatcggctgcatcagcttcaacctgaccaccggagtgtccggagccttctggaccatcgcctacacatcatacaccgaggccctggtgcaggtggagaacacagccataaagaacgtgacctactgcaacagccacatcaacaacatcaagtgctcccagctgacagccaacctgaacaacggcttctacccagtggcctccagcgaggtgggcttcgtgaacaagagcgtggtcctactcccctccttcttcacctacacagcagtcaacatcacaattgacctgggcatgaagctgtccggctacggccagccaatcgccagcaccctgtccaacatcaccctgccaatgcaggacaacaacaccgacgtctactgcatcagaagcaaccagttctccgtgtacgtccactccacctgcaagtcctccctctgggacaacatcttcaaccaggactgcacagacgtgctggaggccacagctgtgatcaagacaggaacctgccctttctcattcgacaagctcaacaactacctgaccttcaacaagttctgcctgagcctgtccccagtgggagccaactgcaagttcgacgtggccgccagaaccaggaccaacgagcaggtggtcagaagcctgtacgtcatctacgaggagggagacaacatcgtgggagtgcccagcgacaactcaggcctgcacgacctgagcgtgctgcacctggactcctgcacagactacaacatctacggcaggacaggagtgggcatcatcaggaggaccaacagcacactgctgtccggcctctactacacctccctgtccggagacttgctgggattcaagaacgtgtcagacggagtcatctacagcgtcaccccatgtgacgtgagcgcccaggcagcagtgatagacggagccatcgtgggagccatgacctcaatcaactcagaactgctgggcctcacccactggacaacaacacccaacttctactactactccatctacaactacacatcagaaagaacaagggacacagcaatcgactccaacgacgtggactgtgagccagtcatcacctactccaacatcggcgtgtgcaagaacggagccctggtgttcatcaacgtcacccactcagacggcgacgtccagccaatctccacaggaaacgtcaccatccccaccaacttcaccatcagcgtgcaggtggagtacatgcaggtctacaccaccccagtctccatcgactgtgccaggtacgtgtgcaacggcaacccaagatgcaacaaactgctgacccagtacgtgagcgcctgccagaccatcgagcaggccctggccatgggcgccaggctggagaacatggaggtggacagcatgctctttgtgagcgagaacgccctgaagcttgccagcgtggaggccttcaacagcaccgaaaacctggactccatctacaaagagtggccctccataggaggctcctggctgggaggcctgaaggacatcctcccatcccacaacagcaaaagaaagtacggcagcgccatcgaagacctgctgttcgacaaggtggtcacctcaggactgggcacagtggacgaggactacaagaggtgcaccggaggctacgacatcgcagacctggtctgtgcccagtactacaacggcatcatggtgctcccaggcgtggccaacgccgacaagatgaccatgtacacagcaagcctggctggaggaatcacactgggagccctgggaggaggggccgtggccattccattcgccgtggccgtgcaggccagactgaactacgtggccctgcagacagacgtgctaaacaagaaccagcagatcctggccaacgccttcaaccaggccatcggcaacatcacccaggccttcggcaaggtgaacgacgcaatccaccagacatcacagggcctggcaacagtggccaaggccctggccaaggtccaggacgtggtgaacacccagggccaggccctctcacacctgacagtccagctgcagaacaacttccaggcaatctcctcctccatctcagacatctacaacagactggaccccccctcagccgacgcccaggtggacagactcatcacaggcaggctgaccgccctcaacgccttcgtgtcccagaccctcaccaggcaggccgaggtgagggccagcaggcagctcgccaaggacaaggtgaacgagtgcgtcagaagccagagccagaggttcggcttctgtggcaacggcacccacctgttctccctggccaacgcagcccccaacggcatgatcttcttccacacagtcctcctcccaacagcatatgagacagtcaccgcctggtcaggaatctgtgcctcagacggggacagaaccttcggcctggtggtcaaggacgtgcagctgacactcttcagaaacctggacgacaaattctacctgacccccaggaccatgtaccagccaagggtggccacctcctcagacttcgtgcagatcgagggctgtgacgtgctcttcgtgaacgccaccgtcatcgacctcccatccatcatcccagactacatcgacatcaaccagacagtgcaggacatcctggagaactaccgccccaactggaccgtgccagagttcaccctagacatattcaacgccacctacctgaacctgacaggagaaattgacgacctggagttcagatcagaaaagctacacaacaccaccgtggagttagccatcctcatagacaacattaacaacaccctcgtcaacctggagtggctcaacaggattgaaacctacgtgaagtggccctggtacgtctggctcctcatcggcctggtggtggtcttctgcatcccactgctgctgttctgctgcttctccaccggctgctgtggatgcatcggctgcctgggctcatgctgccactcaatctgctcaaggaggcagtttgaaaactacgagccaatagaaaaagtccacgtccac

SEQ ID NO: 15 - DNA, 4299 bp, synthetic construct
  source 1..4299: mol_type = other DNA
accacaaataacgagtgcattcaggtcaacgtcacccagctggccggtaacgagaacctaattagagacttcctattctcgaactttaaagaggaaggctctgtggtggtcggaggttactaccccacagaagtgtggtacaattgctcacgtacagccaggaccactgccttccagtacttcaacaacattcatgccttctactttgtcatggaagccatggagaactccactgggaatgccagaggaaagcctctcctcttccatgtccatggagagcctgtctctgtgattatctcagcatatagggatgatgtgcagcagcggccgctgcttaagcatggcctagtgtgcattactaagaaccgacatatcaattatgagcagttcacctccaaccagtggaactccacatgcactggtgctgataggaagatcccgttcagcgttatccccaccgataatggcacaaagatttatggcctagaatggaacgatgattttgttactgcctacatatcaggaagaagttaccacttaaacattaacaccaattggttcaataatgttacacttctgtactctcgcagcagtacggccacttgggagtattcggctgcatatgcctaccaaggtgtaagcaacttcacctactacaagctgaacaatacgaacggtctgaagacttatgagctgtgcgaagactacgagcactgtacgggctatgcgacaaatgtcttcgccccgacgagcggcgggtacataccggatggcttctccttcaacaactggttcctccttaccaatagctccactttcgtatcaggaagatttgttacgaaccaaccccttctcattaactgtctgtggccagtgccctccttcggagtagctgctcaagagttctgtttcgagggtgcacagttcagccagtgtaatggagtgtcgctgaacaacactgtggacgtgatcaggtttaatttgaacttcacagctgatgttcagtccggcatgggcgcgactgtgttcagcctaaacaccacgggtggcgtcatcttggagattagttgttactctgacactgtgtcagagagcagcagttactcctacggagaaattcctttcggcatcacagacggtccccggtactgctatgtgctgtacaacggaactgctttgaagtacctggggacattgccaccttctgtgaaggaaatagccatctctaagtggggtcacttttacattaacggctataatttcttttccactttcccaattggatgcattagcttcaacctgacaacaggtgtgtctggagccttctggaccatcgcctatacctcttacacagaggctctagtacaggtggagaacacagctataaagaacgtgacgtactgtaacagtcacataaacaatatcaagtgttctcagttgactgcgaacttaaacaatgggttttatccagtggcgagctcggaggtggggtttgtaaacaaatctgtggtgctgttgccctccttcttcacgtacactgcagtgaacatcaccattgatttggggatgaaactgtccggctacgggcagcctatagcatctacactgagcaatatcacactgcccatgcaggataacaatacagatgtgtactgtatccgctcaaaccagttctctgtatacgtgcacagtacatgcaagagctcgctatgggacaacattttcaaccaggattgtactgatgtgcttgaagcaactgcagtgatcaaaacaggcacatgcccgttcagctttgataagctcaacaactacctaacgttcaacaagttctgcttgagcctgtctccagtaggcgccaattgcaagtttgacgttgcagcgcgaacacggacaaacgaacaggtagtgcggtcgctctatgttatctacgaggagggggacaacatagtcggggttccatccgacaactcaggtttgcacgacctgagtgtgctccatttggactcatgcacggattataacatctacgggcgcacaggtgtggggataatacgaagaacaaactctacgctattgagcgggctctactacacctcattgagtggggacctgctagggttcaagaacgtatctgacggtgtgatctatagcgtcacaccatgtgacgtatcagcccaagctgctgtgattgacggggcgattgtgggggctatgacttcaattaacagcgagctcctaggcctgacccactggactaccaccccaaacttctactactacagcatttataactataccagtgagcgcaccagggacactgccattgacagcaatgacgtcgactgcgagcctgttattacctacagcaacatcggtgtttgtaagaatggagctctagtcttcataaacgtaacgcactctgatggcgatgttcaaccaatttccactgggaacgtaaccatacccaccaactttactatttccgtccaggtggagtacatgcaagtatataccacgccagtgtccatcgactgcgctcggtatgtgtgcaacggtaacccacgctgcaataagctgctaacgcagtacgtcagcgcctgccagacaatagagcaggcattggcaatgggtgcaaggcttgaaaacatggaggtggactccatgttgttcgtgtctgaaaacgctcttaaactagcatccgtggaggcattcaacagtactgagaacttggactctatctataaggagtggccctccattgggggcagctggcttggaggtctaaaagacatcctgcccagccacaactccaagaggaagtacgggtccgctatagaggacctcctctttgacaaggttgttacttctggtcttggcacagtggacgaagactacaagaggtgcacaggaggctatgatatagctgacctggtgtgtgctcaatactacaacggtataatggttctcccaggtgtggccaacgctgacaagatgacaatgtacacagcctctttagctggaggcattaccctgggagcccttgggggtggcgcagtggcaattccatttgccgttgcggtgcaggcccgactaaactatgtcgcacttcaaacagatgtgctcaacaagaaccaacaaatactggccaacgctttcaaccaggccattggtaacattacgcaggcatttggcaaggtgaatgacgccatccaccagaccagccagggacttgccacagtggccaaggccttggcaaaggtgcaggatgtcgtgaacacacagggtcaggccctctctcatttgacagtgcagcttcagaataacttccaagcaatcagttcaagcatcagcgacatctacaaccggctggaccccccatctgcagatgcgcaggtggacaggctaatcactggacgcttgacggcactaaatgcctttgtcagccaaactctgacccggcaagcagaggtgcgggccagtagacaactggccaaagacaaggtcaacgagtgcgtcaggtcccagtcccagcgttttggattctgtgggaacgggacgcacctgttctcattagccaatgctgcacccaatggcatgatctttttccatactgttctacttcctactgcctatgaaaccgtgaccgcttggagcggcatctgcgcatctgatggcgataggaccttcgggctggtcgttaaggatgtccagctaacgctgttccggaacttggatgacaagttctacctgacccccaggaccatgtaccagccgagagtggcaacgagttctgacttcgtgcaaattgagggctgtgacgtcctgtttgttaatgcaacagtgatcgatctgcccagtatcataccagattacatagacataaaccagacagtccaggacatactggagaattacaggccaaactggaccgtaccagagttcacgctggacatattcaacgctacgtacctcaatttgactggggaaattgatgacttggagttcaggtcggagaagctccacaacaccactgtggagctggccatcctgattgacaacatcaacaacactctggtgaacctggagtggctaaatcgcattgaaacctatgtcaagtggccttggtacgtttggctactgatcggactcgtggtagtcttctgcataccactcctgctattttgctgcttcagcacagggtgctgtggctgcattggatgcctaggttcctgctgtcacagtatctgcagcagaagacaattcgagaactacgagcccatagaaaaggtccacgtacat

SEQ ID NO: 16 - protein, 26 aa, synthetic construct
MRFVMSPTVLLLLLGALAAPQTWAGS

SEQ ID NO: 17 - DNA, 78 bp, synthetic construct
  source 1..78: mol_type = other DNA
atgagatttgtgatgtcccccactgtcctgctgctgctcctgggagccctggcagccccccagacctgggcaggcagc

SEQ ID NO: 18 - DNA, 78 bp, synthetic construct
  source 1..78: mol_type = other DNA
atgagatttgtgatgagccccactgtgctgctgctgctgctgggagccctggcagccccccagacctgggctggctcc

SEQ ID NO: 19 - DNA, 78 bp, synthetic construct
  source 1..78: mol_type = other DNA
atgcgattcgtcatgtcaccaaccgttttactattattactaggagcattagcagcaccgcaaacatgggcaggaagt

SEQ ID NO: 20 - DNA, 78 bp, synthetic construct
  source 1..78: mol_type = other DNA
atgagattcgtgatgtcccctaccgtactactactcctacttggcgcactagcagctcctcaaacttgggccggatcc

SEQ ID NO: 21 - DNA, 78 bp, synthetic construct
  source 1..78: mol_type = other DNA
atgagatttgtgatgagccccactgtgctgctgctgctgctgggagccctggcagccccccagacctgggctggctca

SEQ ID NO: 22 - DNA, 78 bp, synthetic construct
  source 1..78: mol_type = other DNA
atgcgttttgtaatgtcacctactgtactactactactactcggagcactagcagcacctcagacttgggccggatca

SEQ ID NO: 23 - protein, 55 aa, synthetic construct
FLGIIAGVVVLVVTVVVGAVIWRKKCSGRKGPSYSHAARDDSTQGSDSSLMAPKV

SEQ ID NO: 24 - DNA, 165 bp, synthetic construct
  source 1..165: mol_type = other DNA
ttcctgggcatcatcgcaggagtggtggtgctggtggtgaccgtggtggtgggggctgtaatctggaggaagaagtgctcagggagaaagggcccaagctactctcacgccgccagggatgactccacacagggctcagactcctcactgatggctccaaaggtc

SEQ ID NO: 25 - DNA, 165 bp, synthetic construct
  source 1..165: mol_type = other DNA
ttcctgggcatcatcgcaggagtggtggtcctggtggtcacagtcgtggtgggagcagtgatctggaggaagaagtgctcaggaaggaagggcccatcctactcccacgccgccagggacgactcaacccagggctcagacagctccctgatggcccccaaggtg

SEQ ID NO: 26 - DNA, 165 bp, synthetic construct
  source 1..165: mol_type = other DNA
ttcctgggcatcatcgctggcgtggtggtcctggtggtgactgtggtggtcggagccgtcatctggaggaagaagtgcagcggcagaaagggcccaagctacagccacgccgccagagatgacagcacccagggcagcgacagcagcctcatggcccccaaggtc

SEQ ID NO: 27 - DNA, 165 bp, synthetic construct
  source 1..165: mol_type = other DNA
ttcctgggcatcatcgcaggagtggtggtgctggtggtgacagtggtggtgggagcagtgatctggagaaagaaatgcagcgggagaaagggccccagctacagccacgccgccagggacgacagcacccagggcagcgacagcagcctcatggcccccaaggtg

SEQ ID NO: 28 - DNA, 165 bp, synthetic construct
  source 1..165: mol_type = other DNA
ttcctgggcatcatcgccggcgtggtggtcctggtggtgaccgtggtggtcggagcagtgatctggaggaagaagtgctcaggcaggaagggcccatcctacagccacgccgccagagatgacagcacccaaggctcagacagctccctgatggcccccaaggtg

SEQ ID NO: 29 - DNA, 165 bp, synthetic construct
  source 1..165: mol_type = other DNA
ttccttggaatcatagctggggtcgttgtcctcgtagtgactgtagtggtaggcgcagttatctggaggaagaaatgctcggggaggaaagggccctcttacagccatgctgccagggatgactccacacaggggtcagatagcagcctcatggccccaaaggtc

SEQ ID NO: 30 - DNA, 165 bp, synthetic construct
  source 1..165: mol_type = other DNA
ttcctgggcatcatcgccggcgtggtggtcctggtggtcacagtggtggtgggagctgtgatctggagaaagaagtgcagcggcaggaagggcccaagctacagccacgctgccagagatgactccacccagggcagcgacagcagcctgatggcccccaaggtg

SEQ ID NO: 31 - DNA, 165 bp, synthetic construct
  source 1..165: mol_type = other DNA
ttcctgggcataatcgccggcgtggtggtgctggtggtcacagtggtggtcggagcagtgatctggaggaagaagtgctcagggaggaagggcccatcctactcccacgccgccagggacgacagcacccagggctcagactcatccctgatggcccccaaggtg

SEQ ID NO: 32 - DNA, 165 bp, synthetic construct
  source 1..165: mol_type = other DNA
ttcctggggataatcgcaggagtggttgttctagtggtgaccgtggtagttggggcagtgatctggagaaagaaatgctctggccgtaagggaccatcctactcccatgcagcacgtgatgattctacccagggcagcgacagttcattgatggcccctaaagtc

SEQ ID NO: 33 - protein, 27 aa, synthetic construct
YPYDVPDYAYPYDVPDYAYPYDVPDYA

SEQ ID NO: 34 - DNA, 81 bp, synthetic construct
  source 1..81: mol_type = other DNA
tacccctacgatgtgccagactacgcctacccctacgatgtgccagactacgcctacccctacgatgtgccagactacgcc

SEQ ID NO: 35 - DNA, 81 bp, synthetic construct
  source 1..81: mol_type = other DNA
tacccctacgacgtgcccgactacgcctacccctacgacgtgccagactacgcctacccctacgacgtgccagactacgcc

SEQ ID NO: 36 - DNA, 81 bp, synthetic construct
  source 1..81: mol_type = other DNA
tacccatacgatgttccagactacgcttacccatatgacgtgccagactatgcctacccctacgacgtgcccgactacgca

SEQ ID NO: 37 - protein, 6 aa, synthetic construct
HHHHHH

SEQ ID NO: 38 - DNA, 18 bp, synthetic construct
  source 1..18: mol_type = other DNA
caccaccaccaccaccac

SEQ ID NO: 39 - DNA, 18 bp, synthetic construct
  source 1..18: mol_type = other DNA
catcatcatcatcaccac

SEQ ID NO: 40 - protein, 24 aa, synthetic construct
DYKDDDDKDYKDDDDKDYKDDDDK

SEQ ID NO: 41 - DNA, 72 bp, synthetic construct
  source 1..72: mol_type = other DNA
gactacaaagatgatgatgacaaggactacaaagacgacgacgacaaagactacaaggacgatgacgacaag

SEQ ID NO: 42 - DNA, 72 bp, synthetic construct
  source 1..72: mol_type = other DNA
gactacaaggatgatgatgacaaggactacaaagacgacgacgacaaggactacaaggatgacgatgacaag

SEQ ID NO: 43 - DNA, 72 bp, synthetic construct
  source 1..72: mol_type = other DNA
gactataaagacgacgatgacaaagattataaagatgatgacgacaaggactacaaggatgatgatgacaag

SEQ ID NO: 44 - DNA, 68 bp, synthetic construct
  source 1..68: mol_type = other DNA
ggatagctaccagcttacacttgcttctgacacaactgtgttcgctatcaaccacacaaacagacgcc

SEQ ID NO: 45 - DNA, 94 bp, synthetic construct
  source 1..94: mol_type = other DNA
gtgaagccggggcgatcgtcctgagggcccggggcctcttgggctccgggcacccgaacttcctgatctttgaataaagtctgagtgggctgca

SEQ ID NO: 46 - protein, 26 aa, synthetic construct
RAKRGSGATNFSLLKQAGDVEENPGP

SEQ ID NO: 47 - DNA, 78 bp, synthetic construct
  source 1..78: mol_type = other DNA
agagccaagagaggcagcggagccaccaacttcagcctgctgaagcaggccggcgacgtggaggagaacccaggacct

SEQ ID NO: 48 - protein, 15 aa, synthetic construct
GGGGSGGGGSGGGGS

SEQ ID NO: 49 - protein, 45 aa, synthetic construct
GGAGGAGGAGGAAGCGGAGGAGGAGGAAGCGGAGGAGGAGGAAGC